European Patent Specification EP 3 659 614 B9, published October 4, 2023. Title: Oncolytic virus. Applicant: Queen Mary University of London. The sequence listing filed with the application follows.

SEQUENCE LISTING (7 sequences)

SEQ ID NO: 1 - DNA, 70 bp, Artificial sequence
  Synthetic sequence: Modified vaccinia promoter mH5
aaaaattgaaaataaatacaaaggttcttgagggttgtgttaaattgaaagcgagaaataatcataaata

SEQ ID NO: 2 - DNA, 4102 bp, Artificial sequence
  Synthetic sequence: Expression cassette comprising three mH5 promoters
tttggttatactagtatagtcactatcggacaaataaagaaaatcagatgatcgatgaataatacatttaaattcatcatctgtaagatttttgagatgtctcattagaatattattagggttagtactcattatcattcggcagctattacttattttattatttttcaccatatagatcaatcattagatcaaaaattgaaaataaatacaaaggttcttgagggttgtgttaaattgaaagcgagaaataatcataaatagtcgacaatcgaattcccgcggccgggaattcgattagatctaaaaattgaaaataaatacaaaggttcttgagggttgtgttaaattgaaagcgagaaataatcataaatagctaccggactcagatccaccggtcgccaccatggcctcctccgaggacgtcatcaaggagttcatgcgcttcaaggtgcgcatggagggctccgtgaacggccacgagttcgagatcgagggcgagggcgagggccgcccctacgagggcacccagaccgccaagctgaaggtgaccaagggcggccccctgcccttcgcctgggacatcctgtccccccagttccagtacggctccaaggtgtacgtgaagcaccccgccgacatccccgactacaagaagctgtccttccccgagggcttcaagtgggagcgcgtgatgaacttcgaggacggcggcgtggtgaccgtgacccaggactcctccctgcaggacggctccttcatctacaaggtgaagttcatcggcgtgaacttcccctccgacggccccgtaatgcagaagaagactatgggctgggaggcctccaccgagcgcctgtacccccgcgacggcgtgctgaagggcgagatccacaaggccctgaagctgaaggacggcggccactacctggtggagttcaagtccatctacatggccaagaagcccgtgcagctgcccggctactactacgtggactccaagctggacatcacctcccacaacgaggactacactatcgtggagcagtacgagcgcgccgagggccgccaccacctgttcctgtagcggccgcgactctagatcataatcagccataccacatttgtagaggttttacttgctttaaaaaacctcccacacctccccctgaacctgaaacataaaatgaatgcaattgttgttgttaacttgtttattgcagcttataatggttacaaataaagcaatagcatcacaaatttcacaaataaagcatttttttcactgcattctagttgtggtttgtccaaactcatcaatgtatcttaaggcgaaaaattgaaaataaatacaaaggttcttgagggttgtgttaaattgaaagcgagaaataatcataaataaagcttcgaggggctcgcatctctccttcacgcgcccgccgccctacctgaggccgccatccacgccggttgagtcgcgttctgccgcctcccgcctgtggtgcctcctgaactgcgtccgccgtctaggtaagtttaaagctcaggtcgagaccgggcctttgtccggcgctcccttggagcctacctagactcagccggctctccacgctttgcctgaccctgcttgctcaactctacgtctttgtttcgttttctgttctgcgccgttacagatccaagctgtgaccggcgcctacgtaagtgatatctactagatttatcaaaaagagtgttgacttgtgagcgctcacaattgatacttagattcatcgagagggacacgtcgactactaaccttcttctctttcctacagctgagatcaccggcgaaggagggccaccatgggtcaccagcagttggtcatctcttggttttccctggtttttctggcatctcccctcgtggccatatgggaactgaagaaagatgtttatgtcgtagaattggattggtatccggatgcccctggagaaatggtggtcctcacctgtgacacccctgaagaagatggtatcacctggaccttggaccagagcagtgaggtcttaggctctggcaaaaccctgaccatccaagtcaaagagtttggagatgctggccagtacacctgtcacaaaggaggcgaggttctaagccattcgctcctgctgcttcacaaaaaggaagatggaatttggtccactgatattttaaaggaccagaaagaacccaaaaataagacctttctaagatgcgaggccaagaattattctggacgtttcacctgctggtggctgacgacaatcagtactgatttgacattcagtgtcaaaagcagcagaggctcttctgacccccaaggggtgacgtgcggagctgctacactctctgcagagagagtcagaggggacaacaaggagtatgagtactcagtggagtgccaggaggacagtgcctgcccagctgctgaggagagtctgcccattgaggtcatggtggatgccgttcacaagctcaagtatgaaaactacaccagcagcttcttcatcagggacatcatcaaacctgacccacccaagaacttgcagctgaagccattaaagaattctcggcaggtggaggtcagctgggagtaccctgacacctggagtactccacattcctacttctccctgacattctgcgttcaggtccagggcaagagcaagagagaaaagaaagatagagtcttcacggacaagacctcagccacggtcatctgccgcaaaaatgccagcattagcgtgcgggcccaggaccgctactatagctcatcttggagcgaatgggcatctgtgccctgcagtgttcctggagtaggggtacctggggtgggcgccagaaacctccccgtggccactccagacccaggaatgttcccatgccttcaccactcccaaaacctgctgagggccgtcagcaacatgctccagaaggccagacaaactctagaattttacccttgcacttctgaagagattgatcatgaagatatcacaaaagataaaaccagcacagtggaggcctgtttaccattggaattaaccaagaatgagagttgcctaaattccagagagacctctttcataactaatgggagttgcctggcctccagaaagacctcttttatgatggccctgtgccttagtagtatttatgaagacttgaagatgtaccaggtggagttcaagaccatgaatgcaaagctgctgatggatcctaagaggcagatctttctagatcaaaacatgctggcagttattgatgagctgatgcaggccctgaatttcaacagtgagactgtgccacaaaaatcctcccttgaagaaccggatttttataaaactaaaatcaagctctgcatacttcttcatgctttcagaattcgggcagtgactattgatagagtgatgagctatctgaatgcttcctaaaaagcgaggtccctccaaaccgttgtcatttttataaaactttgaaatgaggaaactttgataggatgtggattaagaactagggaggggctagctcgacatgataagatacattgatgagtttggacaaaccacaactagaatgcagtgaaaaaaatgctttatttgtgaaatttgtgatgctattgctttatttgtgaaatttgtgatgctattgctttatttgtaaccattataagctgcaataaacaagttaacaacaacaattgcattcattttatgtttcaggttcagggggaggtgtgggaggttttttaaagcaagtaaaacctctacaaatgtggtagatccatttgggacgcgtatctaataagtagagtcctcatgcttagttaacaactattttttatgttaaatcaattagtacaccgctatgtttaatacttattcatattttagtttttaggattgagaatcaatacaaaaattaatgcatcattaattttagaaatacttagtttccacgtagtcaatgaaacatttgaactcatcgtacaggacgttctcgtacaggacgtaactataaaccggtttatatttgttcaagatagatacaaatccgataactttttttacgaattctacg

SEQ ID NO: 3 - protein, 155 aa, Homo sapiens
MERIVICLMVIFLGTLVHKSSSQGQDRHMIRMRQLIDIVDQLKNYVNDLVPEFLPAPEDVETNCEWSAFSCFQKAQLKSANTGNNERIINVSIKKLKRKPPSTNAGRRQKHRLTCPSCDSYEKKPPKEFLERFKSLLQKMIHQHLSSRTHGSEDS

SEQ ID NO: 4 - protein, 146 aa, Homo sapiens
MERIVICLMVIFLGTLVHKSSSQGQDRHMIRMRQLIDIVDQLKNYVNDLVPEFLPAPEDVETNCEWSAFSCFQKAQLKSANTGNNERIINVSIKKLKRKPPSTNAGRRQKHRLTCPSCDSYEKKPPKEFLERFKSLLQKVSTLSFI

SEQ ID NO: 5 - protein, 219 aa, Homo sapiens
MCPARSLLLVATLVLLDHLSLARNLPVATPDPGMFPCLHHSQNLLRAVSNMLQKARQTLEFYPCTSEEIDHEDITKDKTSTVEACLPLELTKNESCLNSRETSFITNGSCLASRKTSFMMALCLSSIYEDLKMYQVEFKTMNAKLLMDPKRQIFLDQNMLAVIDELMQALNFNSETVPQKSSLEEPDFYKTKIKLCILLHAFRIRAVTIDRVMSYLNAS

SEQ ID NO: 6 - protein, 328 aa, Homo sapiens
MCHQQLVISWFSLVFLASPLVAIWELKKDVYVVELDWYPDAPGEMVVLTCDTPEEDGITWTLDQSSEVLGSGKTLTIQVKEFGDAGQYTCHKGGEVLSHSLLLLHKKEDGIWSTDILKDQKEPKNKTFLRCEAKNYSGRFTCWWLTTISTDLTFSVKSSRGSSDPQGVTCGAATLSAERVRGDNKEYEYSVECQEDSACPAAEESLPIEVMVDAVHKLKYENYTSSFFIRDIIKPDPPKNLQLKPLKNSRQVEVSWEYPDTWSTPHSYFSLTFCVQVQGKSKREKKDRVFTDKTSATVICRKNASISVRAQDRYYSSSWSEWASVPCS

SEQ ID NO: 7 - protein, 144 aa, Homo sapiens
MWLQSLLLLGTVACSISAPARSPSPSTQPWEHVNAIQEARRLLNLSRDTAAEMNETVEVISEMFDLQEPTCLQTRLELYKQGLRGSLTKLKGPLTMMASHYKQHCPPTPETSCATQIITFESFKENLKDFLLVIPFDCWEPVQE